European Patent Specification EP 3 727 462 B1, published November 5, 2025. Title: BICYCLIC PEPTIDE LIGANDS SPECIFIC FOR EphA2. Applicant: BicycleRD Limited. The sequence listing filed with the application follows.

SEQUENCE LISTING (262 sequences)

SEQ ID NO: 1 - protein, 15 aa, Artificial
  Synthetic peptide
ACMNDWLCSLGWTCA

SEQ ID NO: 2 - protein, 14 aa, Artificial
  Synthetic peptide
ACMNDWLCSLGWTC

SEQ ID NO: 3 - protein, 15 aa, Artificial
  Synthetic peptide
ACMNDWLCELGWTCA

SEQ ID NO: 4 - protein, 17 aa, Artificial
  Synthetic peptide
ACTRQGIWCALGFEPCA

SEQ ID NO: 5 - protein, 15 aa, Artificial
  Synthetic peptide
ACMNDWLCTLGWSCA

SEQ ID NO: 6 - protein, 15 aa, Artificial
  Synthetic peptide
ACMNDWLCQLGWTCA

SEQ ID NO: 7 - protein, 15 aa, Artificial
  Synthetic peptide
ACMNDWLCTLGWTCA

SEQ ID NO: 8 - protein, 15 aa, Artificial
  Synthetic peptide
ACMNDWLCDLGWRCA

SEQ ID NO: 9 - protein, 15 aa, Artificial
  Synthetic peptide
ACMNDWLCELGWSCA

SEQ ID NO: 10 - protein, 21 aa, Artificial
  Synthetic peptide
ACRVSPEYCPFGPVWCAGAAA

SEQ ID NO: 11 - protein, 17 aa, Artificial
  Synthetic peptide
ACPWGPAWCPVHGKTCA

SEQ ID NO: 12 - protein, 17 aa, Artificial
  Synthetic peptide
ACPWGPAWCPVNRPGCA

SEQ ID NO: 13 - protein, 21 aa, Artificial
  Synthetic peptide
ACPWGPAWCPVNRPGCAGAAA

SEQ ID NO: 14 - protein, 17 aa, Artificial
  Synthetic peptide
ACPWGPMWCPVNRPGCA

SEQ ID NO: 15 - protein, 17 aa, Artificial
  Synthetic peptide
ACPWGPNWCPVNRPGCA

SEQ ID NO: 16 - protein, 21 aa, Artificial
  Synthetic peptide
AGEMACPWGPFWCPVNRPGCA

SEQ ID NO: 17 - protein, 20 aa, Artificial
  Synthetic peptide
ADVTCPWGPFWCPVNRPGCA

SEQ ID NO: 18 - protein, 21 aa, Artificial
  Synthetic peptide
ADVRTCPWGPFWCPVNRPGCA

SEQ ID NO: 19 - protein, 21 aa, Artificial
  Synthetic peptide
ANDVTCPWGPFWCPVNRPGCA

SEQ ID NO: 20 - protein, 17 aa, Artificial
  Synthetic peptide
ACVPQGIWCALQFEPCA

SEQ ID NO: 21 - protein, 17 aa, Artificial
  Synthetic peptide
ACQKQGLWCALGFEPCA

SEQ ID NO: 22 - protein, 15 aa, Artificial
  Synthetic peptide
ACLVNDDCFYMGLCA

SEQ ID NO: 23 - protein, 13 aa, Artificial
  Synthetic peptide
CANDWLCSLGWTC

SEQ ID NO: 24 - protein, 13 aa, Artificial
  Synthetic peptide
CMNDWLCALGWTC

SEQ ID NO: 25 - protein, 13 aa, Artificial
  Synthetic peptide
CMNDWLCSAGWTC

SEQ ID NO: 26 - protein, 15 aa, Artificial
  Synthetic peptide
ACMNDWLCQLGWKCA

SEQ ID NO: 27 - protein, 16 aa, Artificial
  Synthetic peptide
ACTQNDWLCSLGWTCA

SEQ ID NO: 28 - protein, 17 aa, Artificial
  Synthetic peptide
ACRNIPTMCPFGPVWCA

SEQ ID NO: 29 - protein, 17 aa, Artificial
  Synthetic peptide
ACRVSPEYCPFGPVWCA

SEQ ID NO: 30 - protein, 17 aa, Artificial
  Synthetic peptide
ACRVSPEYCPFGPTWCA

SEQ ID NO: 31 - protein, 17 aa, Artificial
  Synthetic peptide
ACRVSPEYCPFGPSWCA

SEQ ID NO: 32 - protein, 17 aa, Artificial
  Synthetic peptide
ACRVSPEYCPFGPEWCA

SEQ ID NO: 33 - protein, 17 aa, Artificial
  Synthetic peptide
ACRVSPEYCPFGPYWCA

SEQ ID NO: 34 - protein, 17 aa, Artificial
  Synthetic peptide
ACRVSPEYCPFGPLWCA

SEQ ID NO: 35 - protein, 17 aa, Artificial
  Synthetic peptide
ACRVSPEYCPFGPDWCA

SEQ ID NO: 36 - protein, 17 aa, Artificial
  Synthetic peptide
ACPWGPAWCPVRDTNCA

SEQ ID NO: 37 - protein, 17 aa, Artificial
  Synthetic peptide
ACPWGPAWCPVNGARCA

SEQ ID NO: 38 - protein, 16 aa, Artificial
  Synthetic peptide
ACPWGPAWCPVRNPCA

SEQ ID NO: 39 - protein, 16 aa, Artificial
  Synthetic peptide
ACPWGPAWCPVSRVCA

SEQ ID NO: 40 - protein, 15 aa, Artificial
  Synthetic peptide
ACPWGPAWCPVRSCA

SEQ ID NO: 41 - protein, 16 aa, Artificial
  Synthetic peptide
ACPWGPAWCPVKPTCA

SEQ ID NO: 42 - protein, 17 aa, Artificial
  Synthetic peptide
ACPWGPAWCPVNRNGCA

SEQ ID NO: 43 - protein, 21 aa, Artificial
  Synthetic peptide
AVHIPCPWGPSWCPVNRPGCA

SEQ ID NO: 44 - protein, 21 aa, Artificial
  Synthetic peptide
AEGLPCPWGPFWCPVNRPGCA

SEQ ID NO: 45 - protein, 20 aa, Artificial
  Synthetic peptide
ADHACPWGPFWCPVNRPGCA

SEQ ID NO: 46 - protein, 20 aa, Artificial
  Synthetic peptide
ADVHCPWGPFWCPVNRPGCA

SEQ ID NO: 47 - protein, 21 aa, Artificial
  Synthetic peptide
AHDVPCPWGPFWCPVNRPGCA

SEQ ID NO: 48 - protein, 21 aa, Artificial
  Synthetic peptide
ARDDPCPWGPFWCPVNRPGCA

SEQ ID NO: 49 - protein, 17 aa, Artificial
  Synthetic peptide
ACTTGSIWCALQFEPCA

SEQ ID NO: 50 - protein, 17 aa, Artificial
  Synthetic peptide
ACVPQGIWCALRYEPCA

SEQ ID NO: 51 - protein, 17 aa, Artificial
  Synthetic peptide
ACPWGPFWCPVNRPGCA

SEQ ID NO: 52 - protein, 16 aa, Artificial
  Synthetic peptide
ACPWGPFWCPVNRPGC

SEQ ID NO: 53 - protein, 16 aa, Artificial
  Synthetic peptide
  Xaa (3)..(3): Xaa is HyP
ACXWGPFWCPVNRPGC

SEQ ID NO: 54 - protein, 16 aa, Artificial
  Synthetic peptide
  Xaa (3)..(3): Xaa is Aib
ACXWGPFWCPVNRPGC

SEQ ID NO: 55 - protein, 16 aa, Artificial
  Synthetic peptide
  Xaa (3)..(3): Xaa is 4FlPro
ACXWGPFWCPVNRPGC

SEQ ID NO: 56 - protein, 16 aa, Artificial
  Synthetic peptide
  Xaa (4)..(4): Xaa is 1Nal
ACPXGPFWCPVNRPGC

SEQ ID NO: 57 - protein, 16 aa, Artificial
  Synthetic peptide
  Xaa (4)..(4): Xaa is 2Nal
ACPXGPFWCPVNRPGC

SEQ ID NO: 58 - protein, 16 aa, Artificial
  Synthetic peptide
  Xaa (6)..(6): Xaa is Aze
ACPWGXFWCPVNRPGC

SEQ ID NO: 59 - protein, 16 aa, Artificial
  Synthetic peptide
  Xaa (6)..(6): Xaa is HyP
ACPWGXFWCPVNRPGC

SEQ ID NO: 60 - protein, 16 aa, Artificial
  Synthetic peptide
  Xaa (6)..(6): Xaa is Aib
ACPWGXFWCPVNRPGC

SEQ ID NO: 61 - protein, 16 aa, Artificial
  Synthetic peptide
  Xaa (6)..(6): Xaa is 4FlPro
ACPWGXFWCPVNRPGC

SEQ ID NO: 62 - protein, 16 aa, Artificial
  Synthetic peptide
  Xaa (6)..(6): Xaa is Pip
ACPWGXFWCPVNRPGC

SEQ ID NO: 63 - protein, 16 aa, Artificial
  Synthetic peptide
ACPWGPAWCPVNRPGC

SEQ ID NO: 64 - protein, 16 aa, Artificial
  Synthetic peptide
  Xaa (7)..(7): Xaa is 4Pal
ACPWGPXWCPVNRPGC

SEQ ID NO: 65 - protein, 16 aa, Artificial
  Synthetic peptide
  Xaa (7)..(7): Xaa is 4BrPhe
ACPWGPXWCPVNRPGC

SEQ ID NO: 66 - protein, 16 aa, Artificial
  Synthetic peptide
  Xaa (7)..(7): Xaa is 4MeOPhe
ACPWGPXWCPVNRPGC

SEQ ID NO: 67 - protein, 16 aa, Artificial
  Synthetic peptide
  Xaa (7)..(7): Xaa is HPhe
ACPWGPXWCPVNRPGC

SEQ ID NO: 68 - protein, 16 aa, Artificial
  Synthetic peptide
  Xaa (7)..(7): Xaa is 4,4-BPA
ACPWGPXWCPVNRPGC

SEQ ID NO: 69 - protein, 16 aa, Artificial
  Synthetic peptide
  Xaa (7)..(7): Xaa is NO2Phe5
ACPWGPXWCPVNRPGC

SEQ ID NO: 70 - protein, 16 aa, Artificial
  Synthetic peptide
  Xaa (7)..(7): Xaa is 3,4-DCPhe
ACPWGPXWCPVNRPGC

SEQ ID NO: 71 - protein, 16 aa, Artificial
  Synthetic peptide
ACPWGPYWCPVNRPGC

SEQ ID NO: 72 - protein, 16 aa, Artificial
  Synthetic peptide
  Xaa (7)..(7): Xaa is 3PaI
ACPWGPXWCPVNRPGC

SEQ ID NO: 73 - protein, 16 aa, Artificial
  Synthetic peptide
  Xaa (7)..(7): Xaa is Phg
ACPWGPXWCPVNRPGC

SEQ ID NO: 74 - protein, 16 aa, Artificial
  Synthetic peptide
  Xaa (7)..(7): Xaa is 1Nal
ACPWGPXWCPVNRPGC

SEQ ID NO: 75 - protein, 16 aa, Artificial
  Synthetic peptide
  Xaa (7)..(7): Xaa is 2Nal
ACPWGPXWCPVNRPGC

SEQ ID NO: 76 - protein, 16 aa, Artificial
  Synthetic peptide
  Xaa (8)..(8): Xaa is 1Nal
ACPWGPFXCPVNRPGC

SEQ ID NO: 77 - protein, 16 aa, Artificial
  Synthetic peptide
  Xaa (10)..(10): Xaa is Aze
ACPWGPFWCXVNRPGC

SEQ ID NO: 78 - protein, 16 aa, Artificial
  Synthetic peptide
  Xaa (10)..(10): Xaa is HyP
ACPWGPFWCXVNRPGC

SEQ ID NO: 79 - protein, 16 aa, Artificial
  Synthetic peptide
  Xaa (10)..(10): Xaa is 4FlPro
ACPWGPFWCXVNRPGC

SEQ ID NO: 80 - protein, 16 aa, Artificial
  Synthetic peptide
  Xaa (11)..(11): Xaa is tBuGly
ACPWGPFWCPXNRPGC

SEQ ID NO: 81 - protein, 16 aa, Artificial
  Synthetic peptide
ACPWGPFWCPVARPGC

SEQ ID NO: 82 - protein, 16 aa, Artificial
  Synthetic peptide
  Xaa (12)..(12): Xaa is D-Ala
ACPWGPFWCPVXRPGC

SEQ ID NO: 83 - protein, 16 aa, Artificial
  Synthetic peptide
  Xaa (13)..(13): Xaa is HArg
ACPWGPFWCPVNXPGC

SEQ ID NO: 84 - protein, 16 aa, Artificial
  Synthetic peptide
ACPWGPFWCPVNRAGC

SEQ ID NO: 85 - protein, 16 aa, Artificial
  Synthetic peptide
  Xaa (14)..(14): Xaa is D-Ala
ACPWGPFWCPVNRXGC

SEQ ID NO: 86 - protein, 16 aa, Artificial
  Synthetic peptide
  Xaa (14)..(14): Xaa is Aze
ACPWGPFWCPVNRXGC

SEQ ID NO: 87 - protein, 16 aa, Artificial
  Synthetic peptide
  Xaa (14)..(14): Xaa is HyP
ACPWGPFWCPVNRXGC

SEQ ID NO: 88 - protein, 16 aa, Artificial
  Synthetic peptide
  Xaa (14)..(14): Xaa is Pip
ACPWGPFWCPVNRXGC

SEQ ID NO: 89 - protein, 16 aa, Artificial
  Synthetic peptide
  Xaa (14)..(14): Xaa is 4FlPro
ACPWGPFWCPVNRXGC

SEQ ID NO: 90 - protein, 16 aa, Artificial
  Synthetic peptide
  Xaa (14)..(14): Xaa is Aib
ACPWGPFWCPVNRXGC

SEQ ID NO: 91 - protein, 16 aa, Artificial
  Synthetic peptide
ACPWGPFWCPVNRPAC

SEQ ID NO: 92 - protein, 16 aa, Artificial
  Synthetic peptide
  Xaa (15)..(15): Xaa is D-Ala
ACPWGPFWCPVNRPXC

SEQ ID NO: 93 - protein, 16 aa, Artificial
  Synthetic peptide
  Xaa (3)..(3): Xaa is Aib
  Xaa (4)..(4): Xaa is 1Nal2
ACXXGPFWCPVNRPGC

SEQ ID NO: 94 - protein, 16 aa, Artificial
  Synthetic peptide
  Xaa (3)..(3): Xaa is Aib
  Xaa (8)..(8): Xaa is 1Nal
ACXWGPFXCPVNRPGC

SEQ ID NO: 95 - protein, 16 aa, Artificial
  Synthetic peptide
  Xaa (4)..(4): Xaa is 1Nal
  Xaa (12)..(12): Xaa is D-Ala
ACPXGPFWCPVXRPGC

SEQ ID NO: 96 - protein, 16 aa, Artificial
  Synthetic peptide
  Xaa (4)..(4): Xaa is 1Nal
  Xaa (15)..(15): Xaa is D-Ala
ACPXGPFWCPVNRPXC

SEQ ID NO: 97 - protein, 16 aa, Artificial
  Synthetic peptide
  Xaa (8)..(8): Xaa is 1Nal
  Xaa (12)..(12): Xaa is D-Ala
ACPWGPFXCPVXRPGC

SEQ ID NO: 98 - protein, 16 aa, Artificial
  Synthetic peptide
  Xaa (8)..(8): Xaa is 1Nal
  Xaa (15)..(15): Xaa is D-Ala
ACPWGPFXCPVNRPXC

SEQ ID NO: 99 - protein, 16 aa, Artificial
  Synthetic peptide
  Xaa (4)..(4): Xaa is 1Nal
  Xaa (6)..(6): Xaa is Aib
ACPXGXFWCPVNRPGC

SEQ ID NO: 100 - protein, 16 aa, Artificial
  Synthetic peptide
  Xaa (4)..(4): Xaa is 1Nal
  Xaa (8)..(8): Xaa is 1Nal
ACPXGPFXCPVNRPGC

SEQ ID NO: 101 - protein, 16 aa, Artificial
  Synthetic peptide
  Xaa (4)..(4): Xaa is 1Nal
  Xaa (11)..(11): Xaa is tBuGly
ACPXGPFWCPXNRPGC

SEQ ID NO: 102 - protein, 16 aa, Artificial
  Synthetic peptide
  Xaa (4)..(4): Xaa is 1Nal
  Xaa (13)..(13): Xaa is HArg
ACPXGPFWCPVNXPGC

SEQ ID NO: 103 - protein, 16 aa, Artificial
  Synthetic peptide
  Xaa (6)..(6): Xaa is Aib
  Xaa (8)..(8): Xaa is 1Nal
ACPWGXFXCPVNRPGC

SEQ ID NO: 104 - protein, 16 aa, Artificial
  Synthetic peptide
  Xaa (3)..(3): Xaa is Aib
  Xaa (4)..(4): Xaa is 1Nal
  Xaa (12)..(12): Xaa is D-Ala
ACXXGPFWCPVXRPGC

SEQ ID NO: 105 - protein, 16 aa, Artificial
  Synthetic peptide
  Xaa (3)..(3): Xaa is Aib
  Xaa (4)..(4): Xaa is 1Nal
  Xaa (15)..(15): Xaa is D-Ala
ACXXGPFWCPVNRPXC

SEQ ID NO: 106 - protein, 16 aa, Artificial
  Synthetic peptide
  Xaa (4)..(4): Xaa is 1Nal
  Xaa (6)..(6): Xaa is Aib
  Xaa (11)..(11): Xaa is tBuGly
ACPXGXFWCPXNRPGC

SEQ ID NO: 107 - protein, 16 aa, Artificial
  Synthetic peptide
  Xaa (4)..(4): Xaa is 1Nal
  Xaa (6)..(6): Xaa is Aib
  Xaa (12)..(12): Xaa is D-Ala
ACPXGXFWCPVXRPGC

SEQ ID NO: 108 - protein, 16 aa, Artificial
  Synthetic peptide
  Xaa (4)..(4): Xaa is 1Nal
  Xaa (6)..(6): Xaa is Aib
  Xaa (15)..(15): Xaa is D-Ala
ACPXGXFWCPVNRPXC

SEQ ID NO: 109 - protein, 16 aa, Artificial
  Synthetic peptide
  Xaa (4)..(4): Xaa is 1Nal
  Xaa (11)..(11): Xaa is tBuGly
  Xaa (12)..(12): Xaa is D-Ala
ACPXGPFWCPXXRPGC

SEQ ID NO: 110 - protein, 16 aa, Artificial
  Synthetic peptide
  Xaa (4)..(4): Xaa is 1Nal
  Xaa (11)..(11): Xaa is tBuGly
  Xaa (13)..(13): Xaa is HArg
ACPXGPFWCPXNXPGC

SEQ ID NO: 111 - protein, 16 aa, Artificial
  Synthetic peptide
  Xaa (4)..(4): Xaa is 1Nal
  Xaa (11)..(11): Xaa is tBuGly
  Xaa (14)..(14): Xaa is Aib
ACPXGPFWCPXNRXGC

SEQ ID NO: 112 - protein, 16 aa, Artificial
  Synthetic peptide
  Xaa (4)..(4): Xaa ia 1Nal
  Xaa (11)..(11): Xaa ia tBuGly
  Xaa (15)..(15): Xaa ia D-Ala
ACPXGPFWCPXNRPXC

SEQ ID NO: 113 - protein, 16 aa, Artificial
  Synthetic peptide
  Xaa (4)..(4): Xaa is 1Nal
  Xaa (12)..(12): Xaa is D-Ala
  Xaa (13)..(13): Xaa is HArg
ACPXGPFWCPVXXPGC

SEQ ID NO: 114 - protein, 16 aa, Artificial
  Synthetic peptide
  Xaa (4)..(4): Xaa is 1Nal
  Xaa (13)..(13): Xaa is HArg
  Xaa (15)..(15): Xaa is D-Ala
ACPXGPFWCPVNXPXC

SEQ ID NO: 115 - protein, 16 aa, Artificial
  Synthetic peptide
  Xaa (3)..(3): Xaa is Aib
  Xaa (4)..(4): Xaa is 1Nal
  Xaa (6)..(6): Xaa is Aib
  Xaa (14)..(14): Xaa is Aib
ACXXGXFWCPVNRXGC

SEQ ID NO: 116 - protein, 16 aa, Artificial
  Synthetic peptide
  Xaa (4)..(4): Xaa is 1Nal
  Xaa (6)..(6): Xaa is Aib
  Xaa (11)..(11): Xaa is tBuGly
  Xaa (13)..(13): Xaa is HArg
ACPXGXFWCPXNXPGC

SEQ ID NO: 117 - protein, 16 aa, Artificial
  Synthetic peptide
  Xaa (4)..(4): Xaa is 1Nal
  Xaa (6)..(6): Xaa is Aib
  Xaa (11)..(11): Xaa is tBuGly
  Xaa (14)..(14): Xaa is Aib
ACPXGXFWCPXNRXGC

SEQ ID NO: 118 - protein, 16 aa, Artificial
  Synthetic peptide
  Xaa (4)..(4): Xaa is 1Nal
  Xaa (11)..(11): Xaa is tBuGly
  Xaa (13)..(13): Xaa is HArg
  Xaa (14)..(14): Xaa is Aib
ACPXGPFWCPXNXXGC

SEQ ID NO: 119 - protein, 20 aa, Artificial
  Synthetic peptide
  Xaa (2)..(2): Xaa is D-Asp
HXVPCPWGPFWCPVNRPGCA

SEQ ID NO: 120 - protein, 19 aa, Artificial
  Synthetic peptide
  Xaa (2)..(2): Xaa is D-Asp
  Xaa (6)..(6): Xaa is Aib
  Xaa (7)..(7): Xaa is 1Nal
  Xaa (9)..(9): Xaa is Aib
  Xaa (11)..(11): Xaa is 1Nal
  Xaa (14)..(14): Xaa is tBuGly
  Xaa (16)..(16): Xaa is HArg
  Xaa (18)..(18): Xaa is D-Asp
HXVPCXXGXFXCPXNXPXC

SEQ ID NO: 121 - protein, 19 aa, Artificial
  Synthetic peptide
  Xaa (2)..(2): Xaa is D-Asp
  Xaa (6)..(6): Xaa is Aib
  Xaa (7)..(7): Xaa is 1Nal
  Xaa (9)..(9): Xaa is Aib
  Xaa (11)..(11): Xaa is 1Nal
  Xaa (14)..(14): Xaa is tBuGly
  Xaa (17)..(17): Xaa is Aib
  Xaa (18)..(18): Xaa is D-Asp
HXVPCXXGXFXCPXNRXXC

SEQ ID NO: 122 - protein, 20 aa, Artificial
  Synthetic peptide
  Xaa (2)..(2): Xaa is D-Asp
  misc_feature (5)..(5): Xaa can be any naturally occurring amino acid
  Xaa (7)..(7): Xaa is 1Nal
  misc_feature (8)..(8): Xaa can be any naturally occurring amino acid
  Xaa (9)..(9): Xaa is Aib
  misc_feature (10)..(10): Xaa can be any naturally occurring amino acid
  Xaa (11)..(11): Xaa is 1Nal
  misc_feature (12)..(12): Xaa can be any naturally occurring amino acid
  Xaa (14)..(14): Xaa is tBuGly
  misc_feature (15)..(15): Xaa can be any naturally occurring amino acid
  Xaa (16)..(16): Xaa is HArg
  misc_feature (17)..(17): Xaa can be any naturally occurring amino acid
  Xaa (18)..(18): Xaa is D-Asp
  misc_feature (19)..(19): Xaa can be any naturally occurring amino acid
HXVPXCPXGXFXCPXNXPXC

SEQ ID NO: 123 - protein, 19 aa, Artificial
  Synthetic peptide
  Xaa (2)..(2): Xaa is D-Asp
  Xaa (7)..(7): Xaa is 1Nal
  Xaa (9)..(9): Xaa is Aib
  Xaa (11)..(11): Xaa is 1Nal
  Xaa (14)..(14): Xaa is tBuGly
  Xaa (17)..(17): Xaa is Aib
HXVPCPXGXFXCPXNRXGC

SEQ ID NO: 124 - protein, 19 aa, Artificial
  Synthetic peptide
  Xaa (2)..(2): Xaa is D-Asp
  Xaa (7)..(7): Xaa is 1Nal
  Xaa (9)..(9): Xaa is Aib
  Xaa (11)..(11): Xaa is 1Nal
  Xaa (14)..(14): Xaa is tBuGly
  Xaa (17)..(17): Xaa is Aib
  Xaa (18)..(18): Xaa is D-Asp
HXVPCPXGXFXCPXNRXXC

SEQ ID NO: 125 - protein, 19 aa, Artificial
  Synthetic peptide
  Xaa (2)..(2): Xaa is D-Asp
  Xaa (3)..(3): Xaa is C5g
  Xaa (6)..(6): Xaa is Aib
  Xaa (7)..(7): Xaa is 1Nal
  Xaa (9)..(9): Xaa is Aib
  Xaa (11)..(11): Xaa is 1Nal
  Xaa (14)..(14): Xaa is tBuGly
  Xaa (17)..(17): Xaa is Aib
  Xaa (18)..(18): Xaa is D-Asp
HXXPCXXGXFXCPXNRXXC

SEQ ID NO: 126 - protein, 19 aa, Artificial
  Synthetic peptide
  Xaa (2)..(2): Xaa is D-Asp
  Xaa (3)..(3): Xaa is C5g
  Xaa (7)..(7): Xaa is 1Nal
  Xaa (9)..(9): Xaa is Aib
  Xaa (11)..(11): Xaa is 1Nal
  Xaa (14)..(14): Xaa is tBuGly
  Xaa (16)..(16): Xaa is HArg
  Xaa (18)..(18): Xaa is D-Asp
HXXPCPXGXFXCPXNXPXC

SEQ ID NO: 127 - protein, 19 aa, Artificial
  Synthetic peptide
ADVHCPWGPFWCPVNRPGC

SEQ ID NO: 128 - protein, 20 aa, Artificial
  Synthetic peptide
  Xaa (7)..(7): Xaa is 3,3-DPA
ADVHCPXGPFWCPVNRPGCA

SEQ ID NO: 129 - protein, 20 aa, Artificial
  Synthetic Peptide
  Xaa (7)..(7): Xaa is 1Nal
ADVHCPXGPFWCPVNRPGCA

SEQ ID NO: 130 - protein, 20 aa, Artificial
  Synthetic Peptide
ADVHCPWAPFWCPVNRPGCA

SEQ ID NO: 131 - protein, 20 aa, Artificial
  Synthetic peptide
ADVHCPWGAFWCPVNRPGCA

SEQ ID NO: 132 - protein, 20 aa, Artificial
  Synthetic peptide
  Xaa (9)..(9): Xaa is Aib
ADVHCPWGXFWCPVNRPGCA

SEQ ID NO: 133 - protein, 21 aa, Artificial
  Synthetic peptide
ADVHCPWGPFWCAPVNRPGCA

SEQ ID NO: 134 - protein, 20 aa, Artificial
  Synthetic peptide
  Xaa (15)..(15): Xaa is D-Ala
ADVHCPWGPFWCPVXRPGCA

SEQ ID NO: 135 - protein, 20 aa, Artificial
  Synthetic peptide
  Xaa (16)..(16): Xaa is D-Ala
ADVHCPWGPFWCPVNXPGCA

SEQ ID NO: 136 - protein, 19 aa, Artificial
  Synthetic peptide
ADVTCPWGPFWCPVNRPGC

SEQ ID NO: 137 - protein, 19 aa, Artificial
  Synthetic peptide
  Xaa (2)..(2): Xaa is D-Asp
AXVTCPWGPFWCPVNRPGC

SEQ ID NO: 138 - protein, 19 aa, Artificial
  Synthetic peptide
  Xaa (2)..(2): Xaa is D-Asp
  Xaa (3)..(3): Xaa is D-Asp
AXXTCPWGPFWCPVNRPGC

SEQ ID NO: 139 - protein, 19 aa, Artificial
  Synthetic peptide
  Xaa (2)..(2): Xaa is D-Asp
  Xaa (3)..(3): Xaa is Cba
AXXTCPWGPFWCPVNRPGC

SEQ ID NO: 140 - protein, 19 aa, Artificial
  Synthetic peptide
  Xaa (2)..(2): Xaa is D-Asp
  Xaa (3)..(3): Xaa is Cpa
AXXTCPWGPFWCPVNRPGC

SEQ ID NO: 141 - protein, 19 aa, Artificial
  Synthetic peptide
  Xaa (2)..(2): Xaa is D-Asp
  Xaa (3)..(3): Xaa is Cpg
AXXTCPWGPFWCPVNRPGC

SEQ ID NO: 142 - protein, 20 aa, Artificial
  Synthetic peptide
  Xaa (2)..(2): Xaa is D-Asp
  Xaa (3)..(3): Xaa is C5g
AXXVTCPWGPFWCPVNRPGC

SEQ ID NO: 143 - protein, 19 aa, Artificial
  Synthetic peptide
  Xaa (3)..(3): Xaa is tBuGly
ADXTCPWGPFWCPVNRPGC

SEQ ID NO: 144 - protein, 19 aa, Artificial
  Synthetic peptide
  Xaa (2)..(2): Xaa is D-Asp
  Xaa (6)..(6): Xaa is AC3C
AXVTCXWGPFWCPVNRPGC

SEQ ID NO: 145 - protein, 19 aa, Artificial
  Synthetic peptide
  Xaa (2)..(2): Xaa is D-Asp
  Xaa (6)..(6): Xaa is AC4C
AXVTCXWGPFWCPVNRPGC

SEQ ID NO: 146 - protein, 19 aa, Artificial
  Synthetic peptide
  Xaa (2)..(2): Xaa is D-Asp
  Xaa (6)..(6): Xaa is AC5C
AXVTCXWGPFWCPVNRPGC

SEQ ID NO: 147 - protein, 19 aa, Artificial
  Synthetic peptide
  Xaa (2)..(2): Xaa is D-Asp
  Xaa (6)..(6): Xaa is 4BenzylPro
AXVTCXWGPFWCPVNRPGC

SEQ ID NO: 148 - protein, 19 aa, Artificial
  Synthetic peptide
  Xaa (2)..(2): Xaa is D-Asp
  Xaa (6)..(6): Xaa is 4PhenylPro
AXVTCXWGPFWCPVNRPGC

SEQ ID NO: 149 - protein, 19 aa, Artificial
  Synthetic peptide
  Xaa (2)..(2): Xaa is D-Asp
  Xaa (7)..(7): Xaa is 1Nal
AXVTCPXGPFWCPVNRPGC

SEQ ID NO: 150 - protein, 19 aa, Artificial
  Synthetic peptide
  Xaa (2)..(2): Xaa is D-Asp
  Xaa (10)..(10): Xaa is HArg
AXVTCPWGPXWCPVNRPGC

SEQ ID NO: 151 - protein, 19 aa, Artificial
  Synthetic peptide
  Xaa (2)..(2): Xaa is D-Asp
AXVTCPWGPNWCPVNRPGC

SEQ ID NO: 152 - protein, 19 aa, Artificial
  Synthetic peptide
  Xaa (2)..(2): Xaa is D-Asp
AXVTCPWGPAWCPVNRPGC

SEQ ID NO: 153 - protein, 19 aa, Artificial
  Synthetic peptide
  Xaa (2)..(2): Xaa is D-Asp
AXVTCPWGPFWCPLNRPGC

SEQ ID NO: 154 - protein, 19 aa, Artificial
  Synthetic peptide
  Xaa (2)..(2): Xaa is D-Asp
  Xaa (18)..(18): Xaa is D-Asp
AXVTCPWGPFWCPVNRPXC

SEQ ID NO: 155 - protein, 19 aa, Artificial
  Synthetic peptide
  Xaa (2)..(2): Xaa is D-Asp
  Xaa (16)..(16): Xaa is HArg
  Xaa (18)..(18): Xaa is D-Asp
AXVTCPWGPFWCPVNXPXC

SEQ ID NO: 156 - protein, 19 aa, Artificial
  Synthetic peptide
  Xaa (2)..(2): Xaa is D-Asp
  Xaa (16)..(16): Xaa is Aib
  misc_feature (17)..(17): Xaa can be any naturally occurring amino acid
  Xaa (18)..(18): Xaa is D-Asp
AXVTCPWGPFWCPVNRXXC

SEQ ID NO: 157 - protein, 19 aa, Artificial
  Synthetic peptide
  Xaa (2)..(2): Xaa is D-Asp
  Xaa (7)..(7): Xaa is 1Nal
  Xaa (9)..(9): Xaa is Aib
  Xaa (17)..(17): Xaa is Aib
AXVTCPXGXFWCPVNRXGC

SEQ ID NO: 158 - protein, 19 aa, Artificial
  Synthetic peptide
  Xaa (2)..(2): Xaa is D-Asp
  Xaa (9)..(9): Xaa is Aib
  Xaa (11)..(11): Xaa is 1Nal
  Xaa (17)..(17): Xaa is Aib
AXVTCPWGXFXCPVNRXGC

SEQ ID NO: 159 - protein, 19 aa, Artificial
  Synthetic peptide
  Xaa (2)..(2): Xaa is D-Asp
  Xaa (9)..(9): Xaa is Aib
  Xaa (14)..(14): Xaa is tBuGly
  Xaa (17)..(17): Xaa is Aib
AXVTCPWGXFWCPXNRXGC

SEQ ID NO: 160 - protein, 19 aa, Artificial
  Synthetic peptide
  Xaa (2)..(2): Xaa is D-Asp
  Xaa (7)..(7): Xaa is 1Nal
  Xaa (9)..(9): Xaa is Aib
  Xaa (11)..(11): Xaa is 1Nal
  Xaa (17)..(17): Xaa is Aib
AXVTCPXGXFXCPVNRXGC

SEQ ID NO: 161 - protein, 19 aa, Artificial
  Synthetic peptide
  Xaa (2)..(2): Xaa is D-Asp
  Xaa (7)..(7): Xaa is 1Nal
  Xaa (9)..(9): Xaa is Aib
  Xaa (11)..(11): Xaa is 1Nal
  Xaa (14)..(14): Xaa is tBuGly
  Xaa (16)..(16): Xaa is HArg
AXVTCPXGXFXCPXNXPGC

SEQ ID NO: 162 - protein, 19 aa, Artificial
  Synthetic peptide
  Xaa (2)..(2): Xaa is D-Asp
  Xaa (7)..(7): Xaa is 1Nal
  Xaa (9)..(9): Xaa is Aib
  Xaa (11)..(11): Xaa is 1Nal
  Xaa (14)..(14): Xaa is tBuGly
  Xaa (17)..(17): Xaa is Aib
AXVTCPXGXFXCPXNRXGC

SEQ ID NO: 163 - protein, 19 aa, Artificial
  Synthetic peptide
  Xaa (2)..(2): Xaa is D-Asp
  Xaa (7)..(7): Xaa is 1Nal
  Xaa (9)..(9): Xaa is Aib
  Xaa (11)..(11): Xaa is 1Nal
  Xaa (14)..(14): Xaa is tBuGly
  Xaa (16)..(16): Xaa is HArg
  Xaa (18)..(18): Xaa is D-Asp
AXVTCPXGXFXCPXNXPXC

SEQ ID NO: 164 - protein, 18 aa, Artificial
  Synthetic peptide
  Xaa (1)..(1): Xaa is D-Asp
XVTCPWGPFWCPVNRPGC

SEQ ID NO: 165 - protein, 18 aa, Artificial
  Synthetic peptide
  Xaa (1)..(1): Xaa is D-Asp
  Xaa (6)..(6): Xaa is 1Nal
  Xaa (8)..(8): Xaa is Aib
  Xaa (10)..(10): Xaa is 1Nal
  Xaa (13)..(13): Xaa is tBuGly
  Xaa (16)..(16): Xaa is Aib
XVTCPXGXFXCPXNRXGC

SEQ ID NO: 166 - protein, 21 aa, Artificial
  Synthetic peptide
  Xaa (8)..(8): Xaa is 1Nal
AHDVPCPXGPFWCPVNRPGCA

SEQ ID NO: 167 - protein, 20 aa, Artificial
  Synthetic peptide
  Xaa (8)..(8): Xaa is 1Nal
AHDVPCPXGPFWCPVNRPGC

SEQ ID NO: 168 - protein, 20 aa, Artificial
  Synthetic peptide
  Xaa (12)..(12): Xaa is 1Nal
AHDVPCPWGPFXCPVNRPGC

SEQ ID NO: 169 - protein, 20 aa, Artificial
  Synthetic peptide
  Xaa (8)..(8): Xaa is 1Nal
  Xaa (15)..(15): Xaa is tBuGly
AHDVPCPXGPFWCPXNRPGC

SEQ ID NO: 170 - protein, 20 aa, Artificial
  Synthetic peptide
  Xaa (8)..(8): Xaa is 1Nal
  Xaa (10)..(10): Xaa is Aib
  Xaa (15)..(15): Xaa is tBuGly
  Xaa (17)..(17): Xaa is HArg
AHDVPCPXGXFWCPXNXPGC

SEQ ID NO: 171 - protein, 20 aa, Artificial
  Synthetic peptide
  Xaa (8)..(8): Xaa is 1Nal
  Xaa (10)..(10): Xaa is Aib
  Xaa (15)..(15): Xaa is tBuGly
  Xaa (18)..(18): Xaa is Aib
AHDVPCPXGXFWCPXNRXGC

SEQ ID NO: 172 - protein, 20 aa, Artificial
  Synthetic peptide
AHDVPCPWGPFWCPVNRPGC

SEQ ID NO: 173 - protein, 20 aa, Artificial
  Synthetic peptide
  Xaa (1)..(1): Xaa is D-Ala
XHDVPCPWGPFWCPVNRPGC

SEQ ID NO: 174 - protein, 20 aa, Artificial
  Synthetic peptide
AADVPCPWGPFWCPVNRPGC

SEQ ID NO: 175 - protein, 20 aa, Artificial
  Synthetic peptide
  Xaa (2)..(2): Xaa is D-His
AXDVPCPWGPFWCPVNRPGC

SEQ ID NO: 176 - protein, 19 aa, Artificial
  Synthetic peptide
  Xaa (2)..(2): Xaa is D-His
AXDVCPWGPFWCPVNRPGC

SEQ ID NO: 177 - protein, 20 aa, Artificial
  Synthetic peptide
  Xaa (2)..(2): Xaa is D-Ala
AXDVPCPWGPFWCPVNRPGC

SEQ ID NO: 178 - protein, 20 aa, Artificial
  Synthetic peptide
  Xaa (2)..(2): Xaa is D-Asp
AXDVPCPWGPFWCPVNRPGC

SEQ ID NO: 179 - protein, 20 aa, Artificial
  Synthetic peptide
  Xaa (2)..(2): Xaa is Thi
AXDVPCPWGPFWCPVNRPGC

SEQ ID NO: 180 - protein, 20 aa, Artificial
  Synthetic peptide
  Xaa (2)..(2): Xaa is ThiAz
AXDVPCPWGPFWCPVNRPGC

SEQ ID NO: 181 - protein, 20 aa, Artificial
  Synthetic peptide
  Xaa (2)..(2): Xaa is 2FuAla
AXDVPCPWGPFWCPVNRPGC

SEQ ID NO: 182 - protein, 20 aa, Artificial
  Synthetic peptide
  Xaa (2)..(2): Xaa is D-His
  Xaa (4)..(4): Xaa is tBuGly
AXDXPCPWGPFWCPVNRPGC

SEQ ID NO: 183 - protein, 20 aa, Artificial
  Synthetic peptide
AHAVPCPWGPFWCPVNRPGC

SEQ ID NO: 184 - protein, 20 aa, Artificial
  Synthetic peptide
  Xaa (3)..(3): Xaa is D-Ala
AHXVPCPWGPFWCPVNRPGC

SEQ ID NO: 185 - protein, 20 aa, Artificial
  Synthetic peptide
AHEVPCPWGPFWCPVNRPGC

SEQ ID NO: 186 - protein, 20 aa, Artificial
  Synthetic peptide
  Xaa (3)..(3): Xaa is D-Glu
AHXVPCPWGPFWCPVNRPGC

SEQ ID NO: 187 - protein, 20 aa, Artificial
  Synthetic peptide
  Xaa (3)..(3): Xaa is D-Asp
AHXVPCPWGPFWCPVNRPGC

SEQ ID NO: 188 - protein, 20 aa, Artificial
  Synthetic peptide
  Xaa (3)..(3): Xaa is D-Asp
  Xaa (4)..(4): Xaa is tBuGly
AHXXPCPWGPFWCPVNRPGC

SEQ ID NO: 189 - protein, 20 aa, Artificial
  Synthetic peptide
  Xaa (3)..(3): Xaa is D-Asp
  Xaa (5)..(5): Xaa is Sar
AHXVXCPWGPFWCPVNRPGC

SEQ ID NO: 190 - protein, 20 aa, Artificial
  Synthetic peptide
  Xaa (3)..(3): Xaa is D-Asp
  Xaa (5)..(5): Xaa is Aib
AHXVXCPWGPFWCPVNRPGC

SEQ ID NO: 191 - protein, 20 aa, Artificial
  Synthetic peptide
AHDAPCPWGPFWCPVNRPGC

SEQ ID NO: 192 - protein, 20 aa, Artificial
  Synthetic peptide
  Xaa (4)..(4): Xaa is D-Ala
AHDXPCPWGPFWCPVNRPGC

SEQ ID NO: 193 - protein, 20 aa, Artificial
  Synthetic peptide
  Xaa (4)..(4): Xaa is Aib
AHDXPCPWGPFWCPVNRPGC

SEQ ID NO: 194 - protein, 20 aa, Artificial
  Synthetic peptide
  Xaa (4)..(4): Xaa is tBuGly
AHDXPCPWGPFWCPVNRPGC

SEQ ID NO: 195 - protein, 20 aa, Artificial
  Synthetic peptide
AHDVACPWGPFWCPVNRPGC

SEQ ID NO: 196 - protein, 20 aa, Artificial
  Synthetic peptide
  Xaa (5)..(5): Xaa is D-Ala
AHDVXCPWGPFWCPVNRPGC

SEQ ID NO: 197 - protein, 20 aa, Artificial
  Synthetic peptide
  Xaa (5)..(5): Xaa is Aib
AHDVXCPWGPFWCPVNRPGC

SEQ ID NO: 198 - protein, 20 aa, Artificial
  Synthetic peptide
  Xaa (5)..(5): Xaa is Aze
AHDVXCPWGPFWCPVNRPGC

SEQ ID NO: 199 - protein, 20 aa, Artificial
  Synthetic peptide
  Xaa (5)..(5): Xaa is Pip
AHDVXCPWGPFWCPVNRPGC

SEQ ID NO: 200 - protein, 19 aa, Artificial
  Synthetic peptide
HDVPCPWGPFWCPVNRPGC

SEQ ID NO: 201 - protein, 19 aa, Artificial
  Synthetic peptide
  Xaa (1)..(1): Xaa is D-His
XDVPCPWGPFWCPVNRPGC

SEQ ID NO: 202 - protein, 19 aa, Artificial
  Synthetic peptide
  Xaa (2)..(2): Xaa is D-Asp
HXVPCPWGPFWCPVNRPGC

SEQ ID NO: 203 - protein, 20 aa, Artificial
  Synthetic peptide
  Xaa (3)..(3): Xaa is D-Asp
  Xaa (8)..(8): Xaa is 1Nal
  Xaa (15)..(15): Xaa is tBuGly
  Xaa (17)..(17): Xaa is HArg
AHXVPCPXGPFWCPXNXPGC

SEQ ID NO: 204 - protein, 20 aa, Artificial
  Synthetic peptide
  Xaa (2)..(2): Xaa is D-His
  Xaa (11)..(11): Xaa is Psi-Ala
AXDVPCPWGPXWCPVNRPGC

SEQ ID NO: 205 - protein, 20 aa, Artificial
  Synthetic peptide
  Xaa (2)..(2): Xaa is D-His
  Xaa (15)..(15): Xaa is HArg
AXDVPCPWGPFWCPXNRPGC

SEQ ID NO: 206 - protein, 20 aa, Artificial
  Synthetic peptide
  Xaa (2)..(2): Xaa is D-His
  Xaa (8)..(8): Xaa is 1Nal
  Xaa (15)..(15): Xaa is tBuGly
  Xaa (17)..(17): Xaa is HArg
AXDVPCPXGPFWCPXNXPGC

SEQ ID NO: 207 - protein, 20 aa, Artificial
  Synthetic peptide
  Xaa (2)..(2): Xaa is D-His
  Xaa (8)..(8): Xaa is 1Nal
  Xaa (10)..(10): Xaa is Aib
  Xaa (12)..(12): Xaa is 1Nal
  Xaa (15)..(15): Xaa is tBuGly
  Xaa (17)..(17): Xaa is HArg
AXDVPCPXGXFXCPXNXPGC

SEQ ID NO: 208 - protein, 20 aa, Artificial
  Synthetic peptide
  Xaa (2)..(2): Xaa is D-His
  Xaa (8)..(8): Xaa is 1Nal
  Xaa (10)..(10): Xaa is Aib
  Xaa (12)..(12): Xaa is 1Nal
  Xaa (15)..(15): Xaa is tBuGly
  Xaa (18)..(18): Xaa is Aib
AXDVPCPXGXFXCPXNRXGC

SEQ ID NO: 209 - protein, 20 aa, Artificial
  Synthetic peptide
  Xaa (2)..(2): Xaa is D-His
  Xaa (10)..(10): Xaa is Aib
  Xaa (15)..(15): Xaa is tBuGly
  Xaa (18)..(18): Xaa is Aib
AXDVPCPWGXFWCPXNRXGC

SEQ ID NO: 210 - protein, 19 aa, Artificial
  Synthetic peptide
  Xaa (2)..(2): Xaa is D-Asp
  Xaa (6)..(6): Xaa is Aib
  Xaa (7)..(7): Xaa is 1Nal
  Xaa (9)..(9): Xaa is Aib
  Xaa (11)..(11): Xaa is 1Nal
  Xaa (14)..(14): Xaa is tBuGly
HXVPCXXGXFXCPXNRPGC

SEQ ID NO: 211 - protein, 19 aa, Artificial
  Synthetic peptide
  Xaa (2)..(2): Xaa is D-Asp
  Xaa (6)..(6): Xaa is Aib
  Xaa (7)..(7): Xaa is 1Nal
  Xaa (9)..(9): Xaa is Aib
  Xaa (11)..(11): Xaa is 1Nal
  Xaa (14)..(14): Xaa is tBuGly
  Xaa (16)..(16): Xaa is HArg
HXVPCXXGXFXCPXNXPGC

SEQ ID NO: 212 - protein, 19 aa, Artificial
  Synthetic peptide
  Xaa (2)..(2): Xaa is D-Asp
  Xaa (6)..(6): Xaa is Aib
  Xaa (7)..(7): Xaa is 1Nal
  Xaa (9)..(9): Xaa is Aib
  Xaa (11)..(11): Xaa is 1Nal
  Xaa (14)..(14): Xaa is tBuGly
  Xaa (16)..(16): Xaa is HArg
  Xaa (17)..(17): Xaa is Aib
  Xaa (18)..(18): Xaa is D-Asp
HXVPCXXGXFXCPXNXXXC

SEQ ID NO: 213 - protein, 19 aa, Artificial
  Synthetic peptide
  Xaa (2)..(2): Xaa is D-Asp
  Xaa (6)..(6): Xaa is Aib
  Xaa (7)..(7): Xaa is 1Nal
  Xaa (9)..(9): Xaa is Aib
  Xaa (11)..(11): Xaa is 1Nal
  Xaa (14)..(14): Xaa is tBuGly
  Xaa (17)..(17): Xaa is Aib
HXVPCXXGXFXCPXNRXGC

SEQ ID NO: 214 - protein, 19 aa, Artificial
  Synthetic peptide
  Xaa (2)..(2): Xaa is D-Asp
  Xaa (6)..(6): Xaa is Aib
  Xaa (7)..(7): Xaa is 1Nal
  Xaa (9)..(9): Xaa is Aib
  Xaa (14)..(14): Xaa is tBuGly
  Xaa (16)..(16): Xaa is HArg
  Xaa (18)..(18): Xaa is D-Asp
HXVPCXXGXFWCPXNXPXC

SEQ ID NO: 215 - protein, 19 aa, Artificial
  Synthetic peptide
  Xaa (2)..(2): Xaa is D-Asp
  Xaa (6)..(6): Xaa is Aib
  Xaa (7)..(7): Xaa is 1Nal
  Xaa (10)..(10): Xaa is HArg
  Xaa (11)..(11): Xaa is 1Nal
  Xaa (14)..(14): Xaa is tBuGly
  Xaa (17)..(17): Xaa is Aib
HXVPCXXGPXXCPXNRXGC

SEQ ID NO: 216 - protein, 19 aa, Artificial
  Synthetic peptide
  Xaa (2)..(2): Xaa is D-Asp
  Xaa (6)..(6): Xaa is Aib
  Xaa (7)..(7): Xaa is 1Nal
  Xaa (10)..(10): Xaa is HArg
  Xaa (11)..(11): Xaa is 1Nal
  Xaa (14)..(14): Xaa is tBuGly
  Xaa (16)..(16): Xaa is HArg
  Xaa (18)..(18): Xaa is D-Asp
HXVPCXXGPXXCPXNXPXC

SEQ ID NO: 217 - protein, 19 aa, Artificial
  Synthetic peptide
  Xaa (2)..(2): Xaa is D-Asp
  Xaa (6)..(6): Xaa is Aib
  Xaa (10)..(10): Xaa is HArg
  Xaa (11)..(11): Xaa is 1Nal
  Xaa (14)..(14): Xaa is tBuGly
  Xaa (16)..(16): Xaa is HArg
  Xaa (18)..(18): Xaa is D-Asp
HXVPCXWGPXXCPXNXPXC

SEQ ID NO: 218 - protein, 19 aa, Artificial
  Synthetic peptide
  Xaa (2)..(2): Xaa is D-Asp
  Xaa (6)..(6): Xaa is Aib
  Xaa (10)..(10): Xaa is HArg
  Xaa (14)..(14): Xaa is tBuGly
  Xaa (16)..(16): Xaa is HArg
  Xaa (18)..(18): Xaa is D-Asp
HXVPCXWGPXWCPXNXPXC

SEQ ID NO: 219 - protein, 19 aa, Artificial
  Synthetic peptide
  Xaa (2)..(2): Xaa is D-Asp
  Xaa (6)..(6): Xaa is D-Ala
  Xaa (7)..(7): Xaa is 1Nal
  Xaa (9)..(9): Xaa is Aib
  Xaa (11)..(11): Xaa is 1Nal
  Xaa (14)..(14): Xaa is tBuGly
  Xaa (16)..(16): Xaa is HArg
  Xaa (18)..(18): Xaa is D-Asp
HXVPCXXGXFXCPXNXPXC

SEQ ID NO: 220 - protein, 19 aa, Artificial
  Synthetic peptide
  Xaa (2)..(2): Xaa is D-Asp
  Xaa (7)..(7): Xaa is 1Nal
  Xaa (9)..(9): Xaa is Aib
  Xaa (10)..(10): Xaa is HArg
  Xaa (11)..(11): Xaa is 1Nal
  Xaa (14)..(14): Xaa is tBuGly
  Xaa (17)..(17): Xaa is Aib
HXVPCPXGXXXCPXNRXGC

SEQ ID NO: 221 - protein, 19 aa, Artificial
  Synthetic peptide
  Xaa (2)..(2): Xaa is D-Asp
  Xaa (7)..(7): Xaa is 1Nal
  Xaa (9)..(9): Xaa is Aib
  Xaa (10)..(10): Xaa is HArg
  Xaa (11)..(11): Xaa is 1Nal
  Xaa (14)..(14): Xaa is tBuGly
  Xaa (17)..(17): Xaa is Aib
  Xaa (18)..(18): Xaa is D-Asp
HXVPCPXGXXXCPXNRXXC

SEQ ID NO: 222 - protein, 19 aa, Artificial
  Synthetic peptide
  Xaa (2)..(2): Xaa is D-Asp
  Xaa (7)..(7): Xaa is 1Nal
  Xaa (9)..(9): Xaa is Aib
  Xaa (10)..(10): Xaa is HArg
  Xaa (11)..(11): Xaa is 1Nal
  Xaa (14)..(14): Xaa is tBuGly
  Xaa (16)..(16): Xaa is HArg
  Xaa (18)..(18): Xaa is D-Asp
HXVPCPXGXXXCPXNXPXC

SEQ ID NO: 223 - protein, 19 aa, Artificial
  Synthetic peptide
  Xaa (2)..(2): Xaa is D-Asp
  Xaa (7)..(7): Xaa is 1Nal
  Xaa (9)..(9): Xaa is Aib
  Xaa (11)..(11): Xaa is 1Nal
  Xaa (14)..(14): Xaa is tBuGly
HXVPCPXGXFXCPXNRPGC

SEQ ID NO: 224 - protein, 19 aa, Artificial
  Synthetic peptide
  Xaa (2)..(2): Xaa is D-Asp
  Xaa (7)..(7): Xaa is 1Nal
  Xaa (9)..(9): Xaa is Aib
  Xaa (11)..(11): Xaa is 1Nal
  Xaa (14)..(14): Xaa is tBuGly
  Xaa (16)..(16): Xaa is HArg
HXVPCPXGXFXCPXNXPGC

SEQ ID NO: 225 - protein, 19 aa, Artificial
  Synthetic peptide
  Xaa (2)..(2): Xaa is D-Asp
  Xaa (7)..(7): Xaa is 1Nal
  Xaa (9)..(9): Xaa is Aib
  Xaa (11)..(11): Xaa is 1Nal
  Xaa (14)..(14): Xaa is tBuGly
  Xaa (16)..(16): Xaa is HArg
  Xaa (17)..(17): Xaa is Aib
  Xaa (18)..(18): Xaa is D-Asp
HXVPCPXGXFXCPXNXXXC

SEQ ID NO: 226 - protein, 19 aa, Artificial
  Synthetic peptide
  Xaa (2)..(2): Xaa is D-Asp
  Xaa (7)..(7): Xaa is 1Nal
  Xaa (9)..(9): Xaa is Aib
  Xaa (11)..(11): Xaa is 1Nal
  Xaa (17)..(17): Xaa is Aib
HXVPCPXGXFXCPVNRXGC

SEQ ID NO: 227 - protein, 19 aa, Artificial
  Synthetic peptide
  Xaa (2)..(2): Xaa is D-Asp
  Xaa (7)..(7): Xaa is 1Nal
  Xaa (9)..(9): Xaa is Aib
  Xaa (14)..(14): Xaa is tBuGly
  Xaa (16)..(16): Xaa is HArg
  Xaa (18)..(18): Xaa is D-Asp
HXVPCPXGXFWCPXNXPXC

SEQ ID NO: 228 - protein, 19 aa, Artificial
  Synthetic peptide
  Xaa (2)..(2): Xaa is D-Asp
  Xaa (7)..(7): Xaa is 1Nal
  Xaa (9)..(9): Xaa is Aib
  Xaa (17)..(17): Xaa is Aib
HXVPCPXGXFWCPVNRXGC

SEQ ID NO: 229 - protein, 19 aa, Artificial
  Synthetic peptide
  Xaa (2)..(2): Xaa is D-Asp
  Xaa (8)..(8): Xaa is Aza-Gly
HXVPCPWXPFWCPVNRPGC

SEQ ID NO: 230 - protein, 19 aa, Artificial
  Synthetic peptide
  Xaa (2)..(2): Xaa is D-Asp
  Xaa (9)..(9): Xaa is Aib
  Xaa (11)..(11): Xaa is 1Nal
  Xaa (17)..(17): Xaa is Aib
HXVPCPWGXFXCPVNRXGC

SEQ ID NO: 231 - protein, 19 aa, Artificial
  Synthetic peptide
  Xaa (2)..(2): Xaa is D-Asp
  Xaa (9)..(9): Xaa is Aib
  Xaa (11)..(11): Xaa is 1Nal
  Xaa (14)..(14): Xaa is tBuGly
  Xaa (16)..(16): Xaa is HArg
  Xaa (18)..(18): Xaa is D-Asp
HXVPCPWGXFXCPXNXPXC

SEQ ID NO: 232 - protein, 19 aa, Artificial
  Synthetic peptide
  Xaa (2)..(2): Xaa is D-Asp
  Xaa (9)..(9): Xaa is Aib
  Xaa (14)..(14): Xaa is tBuGly
  Xaa (17)..(17): Xaa is Aib
HXVPCPWGXFWCPXNRXGC

SEQ ID NO: 233 - protein, 19 aa, Artificial
  Synthetic peptide
  Xaa (2)..(2): Xaa is D-Asp
  Xaa (9)..(9): Xaa is Aib
  Xaa (14)..(14): Xaa is tBuGly
  Xaa (16)..(16): Xaa is HArg
  Xaa (18)..(18): Xaa is D-Asp
HXVPCPWGXFWCPXNXPXC

SEQ ID NO: 234 - protein, 19 aa, Artificial
  Synthetic peptide
  Xaa (2)..(2): Xaa is D-Asp
  Xaa (10)..(10): Xaa is HArg
  Xaa (14)..(14): Xaa is tBuGly
  Xaa (16)..(16): Xaa is HArg
  Xaa (18)..(18): Xaa is D-Asp
HXVPCPWGPXWCPXNXPXC

SEQ ID NO: 235 - protein, 19 aa, Artificial
  Synthetic peptide
  Xaa (2)..(2): Xaa is D-Asp
  Xaa (3)..(3): Xaa is C5g
  Xaa (6)..(6): Xaa is Aib
  Xaa (9)..(9): Xaa is Aib
  Xaa (14)..(14): Xaa is tBuGly
  Xaa (17)..(17): Xaa is Aib
  Xaa (18)..(18): Xaa is D-Asp
HXXPCXWGXFWCPXNRXXC

SEQ ID NO: 236 - protein, 19 aa, Artificial
  Synthetic peptide
  Xaa (2)..(2): Xaa is D-Asp
  Xaa (3)..(3): Xaa is C5g
  Xaa (7)..(7): Xaa is 1Nal
  Xaa (9)..(9): Xaa is Aib
  Xaa (11)..(11): Xaa is 1Nal
  Xaa (14)..(14): Xaa is tBuGly
  Xaa (17)..(17): Xaa is Aib
HXXPCPXGXFXCPXNRXGC

SEQ ID NO: 237 - protein, 19 aa, Artificial
  Synthetic peptide
  Xaa (2)..(2): Xaa is D-Asp
  Xaa (3)..(3): Xaa is C5g
  Xaa (7)..(7): Xaa is 1Nal
  Xaa (9)..(9): Xaa is Aib
  Xaa (11)..(11): Xaa is 1Nal
  Xaa (14)..(14): Xaa is tBuGly
  Xaa (17)..(17): Xaa is Aib
HXXTCPXGXFXCPXNRXGC

SEQ ID NO: 238 - protein, 19 aa, Artificial
  Synthetic peptide
  Xaa (2)..(2): Xaa is D-Asp
  Xaa (3)..(3): Xaa is C5g
  Xaa (7)..(7): Xaa is 1Nal
  Xaa (9)..(9): Xaa is Aib
  Xaa (11)..(11): Xaa is 1Nal
  Xaa (14)..(14): Xaa is tBuGly
  Xaa (16)..(16): Xaa is HArg
  Xaa (18)..(18): Xaa is D-Asp
HXXTCPXGXFXCPXNXPXC

SEQ ID NO: 239 - protein, 20 aa, Artificial
  Synthetic peptide
  Xaa (2)..(2): Xaa is D-Asp
AXDVTCPWGPFWCPVNRPGC

SEQ ID NO: 240 - protein, 20 aa, Artificial
  Synthetic peptide
  Xaa (2)..(2): Xaa is D-Asp
  Xaa (8)..(8): Xaa is 1Nal
AXDVTCPXGPFWCPVNRPGC

SEQ ID NO: 241 - protein, 20 aa, Artificial
  Synthetic peptide
  Xaa (2)..(2): Xaa is D-Asp
  Xaa (8)..(8): Xaa is 1Nal
  Xaa (12)..(12): Xaa is 1Nal
AXDVTCPXGPFXCPVNRPGC

SEQ ID NO: 242 - protein, 20 aa, Artificial
  Synthetic peptide
  Xaa (2)..(2): Xaa is D-Asp
  Xaa (8)..(8): Xaa is 1Nal
  Xaa (10)..(10): Xaa is Aib
  Xaa (15)..(15): Xaa is tBuGly
  Xaa (17)..(17): Xaa is HArg
AXDVTCPXGXFWCPXNXPGC

SEQ ID NO: 243 - protein, 19 aa, Artificial
  Synthetic peptide
  Xaa (2)..(2): Xaa is D-Asp
  Xaa (7)..(7): Xaa is 1Nal
  Xaa (9)..(9): Xaa is Aib
  Xaa (11)..(11): Xaa is 1Nal
  Xaa (14)..(14): Xaa is tBuGly
  Xaa (17)..(17): Xaa is Aib
HXVTCPXGXFXCPXNRXGC

SEQ ID NO: 244 - protein, 16 aa, Artificial
  Synthetic peptide
ACAWGPFWCPVNRPGC

SEQ ID NO: 245 - protein, 16 aa, Artificial
  Synthetic peptide
ACPAGPFWCPVNRPGC

SEQ ID NO: 246 - protein, 16 aa, Artificial
  Synthetic peptide
ACPWAPFWCPVNRPGC

SEQ ID NO: 247 - protein, 16 aa, Artificial
  Synthetic peptide
ACPWGAFWCPVNRPGC

SEQ ID NO: 248 - protein, 16 aa, Artificial
  Synthetic peptide
ACPWGPFACPVNRPGC

SEQ ID NO: 249 - protein, 16 aa, Artificial
  Synthetic peptide
ACPWGPFWCAVNRPGC

SEQ ID NO: 250 - protein, 16 aa, Artificial
  Synthetic peptide
ACPWGPFWCPANRPGC

SEQ ID NO: 251 - protein, 16 aa, Artificial
  Synthetic peptide
ACPWGPFWCPVNAPGC

SEQ ID NO: 252 - protein, 16 aa, Artificial
  Synthetic peptide
  Xaa (3)..(3): Xaa is D-Ala
ACXWGPFWCPVNRPGC

SEQ ID NO: 253 - protein, 16 aa, Artificial
  Synthetic peptide
  Xaa (4)..(4): Xaa is D-Ala
ACPXGPFWCPVNRPGC

SEQ ID NO: 254 - protein, 16 aa, Artificial
  Synthetic peptide
  Xaa (5)..(5): Xaa is D-Ala
ACPWXPFWCPVNRPGC

SEQ ID NO: 255 - protein, 16 aa, Artificial
  Synthetic peptide
  Xaa (6)..(6): Xaa is D-Ala
ACPWGXFWCPVNRPGC

SEQ ID NO: 256 - protein, 16 aa, Artificial
  Synthetic peptide
  Xaa (7)..(7): Xaa is D-Ala
ACPWGPXWCPVNRPGC

SEQ ID NO: 257 - protein, 16 aa, Artificial
  Synthetic peptide
  Xaa (8)..(8): Xaa is D-Ala
ACPWGPFXCPVNRPGC

SEQ ID NO: 258 - protein, 16 aa, Artificial
  Synthetic peptide
  Xaa (10)..(10): Xaa is D-Ala
ACPWGPFWCXVNRPGC

SEQ ID NO: 259 - protein, 16 aa, Artificial
  Synthetic peptide
  Xaa (11)..(11): Xaa is D-Ala
ACPWGPFWCPXNRPGC

SEQ ID NO: 260 - protein, 16 aa, Artificial
  Synthetic peptide
  Xaa (13)..(13): Xaa is D-Ala
ACPWGPFWCPVNXPGC

SEQ ID NO: 261 - protein, 16 aa, Artificial
  Synthetic peptide
ACPWAPFWCAVNRPGC

SEQ ID NO: 262 - protein, 19 aa, Artificial
  Synthetic peptide
  Xaa (2)..(2): Xaa is D-Asp
  Xaa (7)..(7): Xaa is 1Nal
  Xaa (9)..(9): Xaa is Aib
  Xaa (11)..(11): Xaa is 1Nal
  Xaa (14)..(14): Xaa is tBuGly
  Xaa (17)..(17): Xaa is Aib
  Xaa (18)..(18): Xaa is D-Asp
HXVPCPXAXFXCAXNRXXC